European Patent Application EP 4 155 408 A1, published March 29, 2023. Title: Co-regulatory Sequences Based on Tetracycline and Cumate. Applicant: Shenzhen Eureka Biotechnology Co., LTD. Application EP20936609.5. The sequence listing filed with the application follows.

SEQUENCE LISTING (39 sequences)

SEQ ID NO: 1 - DNA, 1893 bp, Artificial sequence
actgcggccgccctgcaggtcaactagtgacgtcttaattaattgccggctggaacgcgtttcgaacatcgattgaattctggccaagtggatccgctagctctagagtcgacggtaccaagcttgcctcgagccatggagatctgcatgccctaggtccggaaccggttggcgcgccatctggcagcgatcgccgcggaacccctatttgtttatttttctaaatacattcaaatatgtatccgctcatgagacaataaccctgataaatgcttcaataatattgaaaaaggaagagtatgagtattcaacatttccgtgtcgcccttattcccttttttgcggcattttgccttcctgtttttgctcacccagaaacgctggtgaaagtaaaagatgctgaagatcagttgggtgcacgagtgggttacatcgaactggatctcaacagcggtaagatccttgagagttttcgccccgaagaacgttttccaatgatgagcacttttaaagttctgctatgtggcgcggtattatcccgtattgacgccgggcaagagcaactcggtcgccgcatacactattctcagaatgacttggttgagtactcaccagtcacagaaaagcatcttacggatggcatgacagtaagagaattatgcagtgctgccataaccatgagtgataacactgcggccaacttacttctgacaacgatcggaggaccgaaggagctaaccgcttttttgcacaacatgggggatcatgtaactcgccttgatcgttgggaaccggagctgaatgaagccataccaaacgacgagcgtgacaccacgatgcctgtagcaatggcaacaacgttgcgcaaactattaactggcgaactacttactctagcttcccggcaacaattaatagactggatggaggcggataaagttgcaggaccacttctgcgctcggcccttccggctggctggtttattgctgataaatctggagccggtgagcgtgggtctcgcggtatcattgcagcactggggccagatggtaagccctcccgtatcgtagttatctacacgacggggagtcaggcaactatggatgaacgaaatagacagatcgctgagataggtgcctcactgattaagcattggtaacgtacggaagttagagaaaaggcataagtagaaaagatcaaaggatcttcttgagatcctttttttctgcgcgtaatctgctgcttgcaaacaaaaaaaccaccgctaccagcggtggtttgtttgccggatcaagagctaccaactctttttccgaaggtaactggcttcagcagagcgcagataccaaatactgttcttctagtgtagccgtagttaggccaccacttcaagaactctgtagcaccgcctacatacctcgctctgctaatcctgttaccagtggctgctgccagtggcgataagtcgtgtcttaccgggttggactcaagacgatagttaccggataaggcgcagcggtcgggctgaacggggggttcgtgcacacagcccagcttggagcgaacgacctacaccgaactgagatacctacagcgtgagctatgagaaagcgccacgcttcccgaagggagaaaggcggacaggtatccggtaagcggcagggtcggaacaggagagcgcacgagggagcttccagggggaaacgcctggtatctttatagtcctgtcgggtttcgccacctctgacttgagcgtcgatttttgtgatgctcgtcaggggggcggagcctatggaaaaacgccagcaacgcggcctttttacggttcctggccttttgctggccttttgctcatctcatgaaaattatgcaaattgagccagtcaggcagt

SEQ ID NO: 2 - DNA, 2900 bp, Artificial sequence
gcggccgcatctatacagttgaagtcggaagtttacatacacttaagttggagtcattaaaactcgtttttcaactactccacaaatttcttgttaacaaacaatagttttggcaagtcagttaggacatctactttgtgcatgacacaagtcatttttccaacaattgtttacagacagattatttcacttataattcactgtatcacaattccagtgggtcagaagtttacatacactaagttgactgtgcctttaaacagcttggaaaattccagaaaatgatgtcatggctttagcctgcagggagggacagcccccccccaaagcccccagggatgtaattacgtccctcccccgctagggggcagcagcgagccgcccggggctccgctccggtccggcgctccccccgcatccccgagccggcagcgtgcggggacagcccgggcacggggaaggtggcacgggatcgctttcctctgaacgcttctcgctgctctttgagcctgcagacacctggggggatacggggaaaaggacctgcaggtcaactagtgacgtcttaattaattgccggctggacgtacgcgtctagttattaatagtaatcaattacggggtcattagttcatagcccatatatggagttccgcgttacataacttacggtaaatggcccgcctggctgaccgcccaacgacccccgcccattgacgtcaataatgacgtatgttcccatagtaacgccaatagggactttccattgacgtcaatgggtggagtatttacggtaaactgcccacttggcagtacatcaagtgtatcatatgccaagtacgccccctattgacgtcaatgacggtaaatggcccgcctggcattatgcccagtacatgaccttatgggactttcctacttggcagtacatctacgtattagtcatcgctattaccatggtgatgcggttttggcagtacatcaatgggcgtggatagcggtttgactcacggggatttccaagtctccaccccattgacgtcaatgggagtttgttttggcaccaaaatcaacgggactttccaaaatgtcgtaacaactccgccccattgacgcaaatgggcggtaggcgtgtacggtgggaggtctatataagcagagctcgtttagtgaaccgtcagatcgcctggagacgccatccacgctgttttgacctccatagaagacaccgggaccgatccagcctccgcggattcgaatcccggccgggaacggtgcattggaacgcggattccccgtgccaagagtgacgtaagtaccgcctatagagtctataggcccacaaaaaatgctttcttcttttaatatacttttttgtttatcttatttctaatactttccctaatctctttctttcagggcaataatgatacaatgtatcatgcctctttgcaccattctaaagaataacagtgataatttctgggttaaggcaatagcaatatttctgcatataaatatttctgcatataaattgtaactgatgtaagaggtttcatattgctaatagcagctacaatccagctaccattctgcttttattttatggttgggataaggctggattattctgagtccaagctaggcccttttgctaatcatgttcatacctcttatcttcctcccacagctcctgggcaacgtgctggtctgtgtgctggcccatcactttggcaaagaattgggattcgaacatcgattgaattctggccaggatccgctagctctagagtcgacggtaccagtactaagcttgcctcgagccatggagatctacgggtggcatccctgtgacccctccccagtgcctctcctggccctggaagttgccactccagtgcccaccagccttgtcctaataaaattaagttgcatcattttgtctgactaggtgtccttctataatattatggggtggaggggggtggtatggagcaaggggcaagttgggaagacaacctgtagggcctgcggggtctattgggaaccaagctggagtgcagtggcacaatcttggctcactgcaatctccgcctcctgggttcaagcgattctcctgcctcagcctcccgagttgttgggattccaggcaagcatgaccaggctcagctaatttttgtttttttggtagagacggggtttcaccatattggccaggctggtctccaactcctaatctcaggtgatctacccaccttggcctcccaaattgctgggattacaggcgtgaaccactgctcccttccctgtccttgcatgccctaggcagctgtccggaaccggtgtttaaacaggccttttccccgtatccccccaggtgtctgcaggctcaaagagcagcgagaagcgttcagaggaaagcgatcccgtgccaccttccccgtgcccgggctgtccccgcacgctgccggctcggggatgcggggggagcgccggaccggagcggagccccgggcggctcgctgctgccccctagcgggggagggacgtaattacatccctgggggctttgggggggggctgtccctcaggccttggcgcgccctaaagccatgacatcattttctggaattttccaagctgtttaaaggcacagtcaacttagtgtatgtaaacttctgacccactggaattgtgatacagtgaattataagtgaaataatctgtctgtaaacaattgttggaaaaatgacttgtgtcatgcacaaagtagatgtcctaactgacttgccaaaactattgtttgttaacaagaaatttgtggagtagttgaaaaacgagttttaatgactccaacttaagtgtatgtaaacttccgacttcaactgtatagcgatcgc

SEQ ID NO: 3 - DNA, 1208 bp, Artificial sequence
actagtgtgtgtcagttagggtgtggaaagtccccaggctccccagcaggcagaagtatgcaaagcatgcatctcaattagtcagcaaccaggtgtggaaagtccccaggctccccagcaggcagaagtatgcaaagcatgcatctcaattagtcagcaaccatagtcccgcccctaactccgcccatcccgcccctaactccgcccagttccgcccattctccgccccatggctgactaattttttttatttatgcagaggccgaggccgcctctgcctctgagctattccagaagtagtgaggaggcttttttggaggccataggcttttgcaaaaagctatggtgagcaagggcgaggagctgttcaccggggtggtgcccatcctggtcgagctggacggcgacgtaaacggccacaagttcagcgtgtccggcgagggcgagggcgatgccacctacggcaagctgaccctgaagttcatctgcaccaccggcaagctgcccgtgccctggcccaccctcgtgaccaccctgacctacggcgtgcagtgcttcagccgctaccccgaccacatgaagcagcacgacttcttcaagtccgccatgcccgaaggctacgtccaggagcgcaccatcttcttcaaggacgacggcaactacaagacccgcgccgaggtgaagttcgagggcgacaccctggtgaaccgcatcgagctgaagggcatcgacttcaaggaggacggcaacatcctggggcacaagctggagtacaactacaacagccacaacgtctatatcatggccgacaagcagaagaacggcatcaaggtgaacttcaagatccgccacaacatcgaggacggcagcgtgcagctcgccgaccactaccagcagaacacccccatcggcgacggccccgtgctgctgcccgacaaccactacctgagcacccagtccgccctgagcaaagaccccaacgagaagcgcgatcacatggtcctgctggagttcgtgaccgccgccgggatcactctcggcatggacgagctgtacaagtaaaacttgtttattgcagcttataatggttacaaataaagcaatagcatcacaaatttcacaaataaagcatttttttcactgcattctagttgtggtttgtccaaactcatcaatgtatcttacctaggcagctgtccggaaccggt

SEQ ID NO: 4 - DNA, 908 bp, Artificial sequence
acgcgttactccctatcagtgatagagaacgtatgaagagtttactccctatcagtgatagagaacgtatgcagactttactccctatcagtgatagagaacgtataaggagtttactccctatcagtgatagagaacgtatgaccagtttactccctatcagtgatagagaacgtatctacagtttactccctatcagtgatagagaacgtatatccagtttactccctatcagtgatagagaacgtattaggcgtgtacggtgggcgcctataaaagcagagctcgtttagtgaaccgtcagatcgcctggagcaattccacatacaaacagaccagattgtctgtttgttacacttttgtcttataccaactttccgtaccacttcctaccctcgtaaattcgaatcccggccgggaacggtgcattggaacgcggattccccgtgccaagagtgacgtaagtaccgcctatagagtctataggcccacaaaaaatgctttcttcttttaatatacttttttgtttatcttatttctaatactttccctaatctctttctttcagggcaataatgatacaatgtatcatgcctctttgcaccattctaaagaataacagtgataatttctgggttaaggcaatagcaatatttctgcatataaatatttctgcatataaattgtaactgatgtaagaggtttcatattgctaatagcagctacaatccagctaccattctgcttttattttatggttgggataaggctggattattctgagtccaagctaggcccttttgctaatcatgttcatacctcttatcttcctcccacagctcctgggcaacgtgctggtctgtgtgctggcccatcactttggcaaagaattgggattcgaaatcgat

SEQ ID NO: 5 - DNA, 880 bp, Artificial sequence
acgcgttactccctatcagtgatagagaacgtatgaagagtttactccctatcagtgatagagaacgtatgcagactttactccctatcagtgatagagaacgtataaggagtttactccctatcagtgatagagaacgtatgaccagtttactccctatcagtgatagagaacgtatctacagtttactccctatcagtgatagagaacgtatatccagtttactccctatcagtgatagagaacgtattaggcgtgtacggtgggcgcctataaaagcagagctcgtttagtgaaccgtcagatcgcctggagcaattccacaacacttttgtcttataccaactttccgtaccacttcctaccctcgtaaattcgaatcccggccgggaacggtgcattggaacgcggattccccgtgccaagagtgacgtaagtaccgcctatagagtctataggcccacaaaaaatgctttcttcttttaatatacttttttgtttatcttatttctaatactttccctaatctctttctttcagggcaataatgatacaatgtatcatgcctctttgcaccattctaaagaataacagtgataatttctgggttaaggcaatagcaatatttctgcatataaatatttctgcatataaattgtaactgatgtaagaggtttcatattgctaatagcagctacaatccagctaccattctgcttttattttatggttgggataaggctggattattctgagtccaagctaggcccttttgctaatcatgttcatacctcttatcttcctcccacagctcctgggcaacgtgctggtctgtgtgctggcccatcactttggcaaagaattgggattcgaaatcgat

SEQ ID NO: 6 - DNA, 890 bp, Artificial sequence
acgcgtgacgaggatcgttcgagcgagtttactccctatcagtgatagagaacgtatgtcgagtttactccctatcagtgatagagaacgatgtcgagtttactccctatcagtgatagagaacgtatgtcgagtttactccctatcagtgatagagaacgtatgtcgagtttactccctatcagtgatagagaacgtatgtcgagtttatccctatcagtgatagagaacgtatgtcgagtttactccctatcagtgatagagaacgtatgtcgaggtaggcgtgtacggtgggaggcctatataagcaaccggtgtttagtgaaccgtcagatcgcctggagacgccatcataatacaaacagaccagattgtctgtttgttttcgaatcccggccgggaacggtgcattggaacgcggattccccgtgccaagagtgacgtaagtaccgcctatagagtctataggcccacaaaaaatgctttcttcttttaatatacttttttgtttatcttatttctaatactttccctaatctctttctttcagggcaataatgatacaatgtatcatgcctctttgcaccattctaaagaataacagtgataatttctgggttaaggcaatagcaatatttctgcatataaatatttctgcatataaattgtaactgatgtaagaggtttcatattgctaatagcagctacaatccagctaccattctgcttttattttatggttgggataaggctggattattctgagtccaagctaggcccttttgctaatcatgttcatacctcttatcttcctcccacagctcctgggcaacgtgctggtctgtgtgctggcccatcactttggcaaagaattgggattcgaaatcgat

SEQ ID NO: 7 - DNA, 845 bp, Artificial sequence
acgcgtgacgaggatcgttcgagcgagtttactccctatcagtgatagagaacgtatgtcgagtttactccctatcagtgatagagaacgatgtcgagtttactccctatcagtgatagagaacgtatgtcgagtttactccctatcagtgatagagaacgtatgtcgagtttactccctatcagtgatagagaacgtatgtcgagtttatccctatcagtgatagagaacgtatgtcgagtttactccctatcagtgatagagaacgtatgtcgaggtaggcgtgtacggtgggaggcctatataagcagagctcgtttagtgaaccgtcagatcgccttcgaatcccggccgggaacggtgcattggaacgcggattccccgtgccaagagtgacgtaagtaccgcctatagagtctataggcccacaaaaaatgctttcttcttttaatatacttttttgtttatcttatttctaatactttccctaatctctttctttcagggcaataatgatacaatgtatcatgcctctttgcaccattctaaagaataacagtgataatttctgggttaaggcaatagcaatatttctgcatataaatatttctgcatataaattgtaactgatgtaagaggtttcatattgctaatagcagctacaatccagctaccattctgcttttattttatggttgggataaggctggattattctgagtccaagctaggcccttttgctaatcatgttcatacctcttatcttcctcccacagctcctgggcaacgtgctggtctgtgtgctggcccatcactttggcaaagaattgggattcgaaatcgat

SEQ ID NO: 8 - DNA, 414 bp, Artificial sequence
acgcgttactccctatcagtgatagagaacgtatgaagagtttactccctatcagtgatagagaacgtatgcagactttactccctatcagtgatagagaacgtataaggagtttactccctatcagtgatagagaacgtatgaccagtttactccctatcagtgatagagaacgtatctacagtttactccctatcagtgatagagaacgtatatccagtttactccctatcagtgatagagaacgtattaggcgtgtacggtgggcgcctataaaagcagagctcgttacaaacagaccagattgtctgtttgttttagtgaaccgtcagatcgcctggagcaattccacaacacttttgtcttataccaactttccgtaccacttcctaccctcgtaaattcgaaatcgat

SEQ ID NO: 9 - DNA, 414 bp, Artificial sequence
acgcgttactccctatcagtgatagagaacgtatgaagagtttactccctatcagtgatagagaacgtatgcagactttactccctatcagtgatagagaacgtataaggagtttactccctatcagtgatagagaacgtatgaccagtttactccctatcagtgatagagaacgtatctacagtttactccctatcagtgatagagaacgtatatccagtttactccctatcagtgatagagaacgtattaggcgtgtacggtgggcgcctataaaagcagagctcgtttagtgaaccgtcagatacaaacagaccagattgtctgtttgtttcgcctggagcaattccacaacacttttgtcttataccaactttccgtaccacttcctaccctcgtaaattcgaaatcgat

SEQ ID NO: 10 - DNA, 415 bp, Artificial sequence
acgcgttactccctatcagtgatagagaacgtatgaagagtttactccctatcagtgatagagaacgtatgcagactttactccctatcagtgatagagaacgtataaggagtttactccctatcagtgatagagaacgtatgaccagtttactccctatcagtgatagagaacgtatctacagtttactccctatcagtgatagagaacgtatatccagtttactccctatcagtgatagagaacgtattaggcgtgtacggtgggcgcctataaaagcagagctcgtttagtgaaccgtcagatcgcctggagcaattccacaacacttttgtcttataccaactttccgtaccacttcctaccctcgtaaaatacaaacagaccagattgtctgtttgttttcgaaatcgat

SEQ ID NO: 11 - DNA, 472 bp, Artificial sequence
acgcgttactccctatcagtgatagagaacgtatgaagagtttactccctatcagtgatagagaacgtatgcagactttactccctatcagtgatagagaacgtataaggagtttactccctatcagtgatagagaacgtatgaccagtttactccctatcagtgatagagaacgtatctacagtttactccctatcagtgatagagaacgtatatccagtttactccctatcagtgatagagaacgtattaggcgtgtacggtgggcgcctataaaagcagagctcgtttagtgaaccgtcagatcgcctggagcaattccacatacaaacagaccagattgtctgtttgttttcgatattaggatatcactccgtttaaactacaaacagaccagattgtctgtttgttacacttttgtcttataccaactttccgtaccacttcctaccctcgtaaattcgaaatcgat

SEQ ID NO: 12 - DNA, 588 bp, Artificial sequence
acgcgttactccctatcagtgatagagaacgtatgaagagtttactccctatcagtgatagagaacgtatgcagactttactccctatcagtgatagagaacgtataaggagtttactccctatcagtgatagagaacgtatgaccagtttactccctatcagtgatagagaacgtatctacagtttactccctatcagtgatagagaacgtatatccagtttactccctatcagtgatagagaacgtattaggcgtgtacggtgggcgcctataaaagcagagctcgtttagtgaaccgtcagatcgcctggagcaattccacatacaaacagaccagattgtctgtttgttttcgatattaggatatcgtgtgcatcaaagtacaaacagaccagattgtctgtttgttcagctgcatgcatctcaattagtcagcaactacaaacagaccagattgtctgtttgttggcagaagtatgatatcactccgtttaaactacaaacagaccagattgtctgtttgttacacttttgtcttataccaactttccgtaccacttcctaccctcgtaaattcgaaatcgat

SEQ ID NO: 13 - DNA, 704 bp, Artificial sequence
acgcgttactccctatcagtgatagagaacgtatgaagagtttactccctatcagtgatagagaacgtatgcagactttactccctatcagtgatagagaacgtataaggagtttactccctatcagtgatagagaacgtatgaccagtttactccctatcagtgatagagaacgtatctacagtttactccctatcagtgatagagaacgtatatccagtttactccctatcagtgatagagaacgtattaggcgtgtacggtgggcgcctataaaagcagagctcgtttagtgaaccgtcagatcgcctggagcaattccacatacaaacagaccagattgtctgtttgttttcgatattaggatatcgtgtgcatcaaagtacaaacagaccagattgtctgtttgttcagctgcaacatgccttacaaggagagaaatacaaacagaccagattgtctgtttgttcctaggtttatatagtgaatagagttaggctacaaacagaccagattgtctgtttgttcagctgcatgcatctcaattagtcagcaactacaaacagaccagattgtctgtttgttggcagaagtatgatatcactccgtttaaactacaaacagaccagattgtctgtttgttacacttttgtcttataccaactttccgtaccacttcctaccctcgtaaattcgaaatcgat

SEQ ID NO: 14 - DNA, 210 bp, Artificial sequence
gtcaatcgatgctgccgcagcaaaagcaggagcagatgccgccgtcgcaggcgaagatgtcgcagacggaggaggcgatgctgccggcggaggaggcgaagtaagtagagggctgggctgggctgtggggggtgtggggtgcgggactgggcagtctgggagtccctctcaccacttttcttacctttctaggatgctgccggatccgac

SEQ ID NO: 15 - DNA, 633 bp, Artificial sequence
atcgatgccaccatgtctccaaagaggagaacccaggcagagagggcaatggagacacagggcaagctgatcgccgccgccctgggcgtgctgagggagaagggatacgcaggcttccgcatcgccgatgtgccaggagccgccggcgtgtcccggggcgcacagtctcaccacttccctaccaagctggagctgctgctggccacatttgagtggctgtatgagcagatcaccgagaggagccgcgccaggctggcaaagctgaagccagaggacgatgtgatccagcagatgctggacgatgccgccgagttctttctggacgatgactttagcatctccctggatctgatcgtggccgccgatagagaccccgccctgagggagggcatccagaggacagtggagagaaacaggttcgtggtggaggatatgtggctgggcgtgctggtgtctcgcggcctgagccgggatgacgcagaggacatcctgtggctgatctttaacagcgtgcggggcctggccgtgagatccctgtggcagaaggacaaggagcggttcgagcgcgtgcggaattccaccctggagatcgccagagagaggtacgccaagtttaagagatgataactcgag

SEQ ID NO: 16 - DNA, 1496 bp, Artificial sequence
actagtgtgtgtcagttagggtgtggaaagtccccaggctccccagcaggcagaagtatgcaaagcatgcatctcaattagtcagcaaccaggtgtggaaagtccccaggctccccagcaggcagaagtatgcaaagcatgcatctcaattagtcagcaaccatagtcccgcccctaactccgcccatcccgcccctaactccgcccagttccgcccattctccgccccatggctgactaattttttttatttatgcagaggccgaggccgcctctgcctctgagctattccagaagtagtgaggaggcttttttggaggccataggcttttgcaaaaagctatgaaaaagcctgaactcacagcgacttctgttgagaagtttctgatcgaaaagttcgacagcgttagcgacctgatgcagctctcggagggcgaggaatctagggctttcagcttcgatgtaggagggcgtggatatgtcctgcgggtaaatagctgcgccgatggtttctacaaagatcgttatgtttatcggcactttgcatcggctgcgctcccgattcccgaagtgcttgacattggggagttcagcgagagcctgacctattgcatctcccgccgcgcacagggcgtaactttgcaagacctccctgaaaccgaactgcccgctgttctacaacctgtcgcggaggctatggacgctattgctgctgccgatctttcccagacttccgggttcggcccatttggaccgcaaggaatcggtcaatacactacatggcgtgatttcatttgcgcgattgctgatccccatgtgtatcattggcaaactgtgatggatgataccgtcagcgcgagtgtcgcgcaggctctcgatgagctgatgctttgggccgaggattgccccgaagttcgccacttggtccacgcggatttcggcagcaacaatgtcctgacagataatggccgcataacagcggtcattgattggagcgaagctatgttcggggattcccaatacgaggtcgctaacatctttttctggcgtccttggttggcttgtatggagcagcaaacgcgctactttgaaagacgacatccagagcttgcaggatcgcctcggctccgggcgtatatgctccgcattggtcttgaccaactctatcagagcttggtggacggcaatttcgatgatgctgcttgggcgcagggtcgatgtgatgcaatcgtccgaagtggagccgggactgtcgggcgaacacaaatcgcccgcagaagcgcagccgtctggaccgatggctgtgtagaagttctcgccgatagtggaaacagacgcccctctactcgtccgagggcaaaggaatagaacttgtttattgcagcttataatggttacaaataaagcaatagcatcacaaatttcacaaataaagcatttttttcactgcattctagttgtggtttgtccaaactcatcaatgtatcttaaccggt

SEQ ID NO: 17 - DNA, 1979 bp, Artificial sequence
acgcgtgacattgattattgacatgttattaatagtaatcaattacggggtcattagttcatagcccatatatggagttccgcgttacataacttacggtaaatggcccgcctggctgaccgcccaacgacccccgcccattgacgtcaataatgacgtatgttcccatagtaacgccaatagggactttccattgacgtcaatgggtggagtatttacggtaaactgcccacttggcagtacatcaagtgtatcatatgccaagtacgccccctattgacgtcaatgacggtaaatggcccgcctggcattatgcccagtacatgaccttatgggactttcctacttggcagtacatctacgtattagtcatcgctattaccatggtcgaggtgagccccacgttctgcttcactctccccatctcccccccctccccacccccaattttgtatttatttattttttaattattttgtgcagcgatgggggcggggggggggggggggcgcgcgccaggcggggcggggcggggcgaggggcggggcggggcgaggcggagaggtgcggcggcagccaatcagagcggcgcgctccgaaagtttccttttatggcgaggcggcggcggcggcggccctataaaaagcgaagcgcgcggcgggcgttcgaaggagtcgctgcgacgctgccttcgccccgtgccccgctccgccgccgcctcgcgccgcccgccccggctctgactgaccgcgttactcccacaggtgagcgggcgggacggcccttctcctccgggctgtaattagcgcttggtttaatgacggcttgtttcttttctgtggctgcgtgaaagccttgaggggctccgggagggccctttgtgcggggggagcggctcggggggtgcgtgcgtgtgtgtgtgcgtggggagcgccgcgtgcggctccgcgctgcccggcggctgtgagcgctgcgggcgcggcgcggggctttgtgcgctccgcagtgtgcgcgaggggagcgcggccgggggcggtgccccgcggtgcggggggggctgcgaggggaacaaaggctgcgtgcggggtgtgtgcgtgggggggtgagcagggggtgtgggcgcgtcggtcgggctgcaaccccccctgcacccccctccccgagttgctgagcacggcccggcttcgggtgcggggctccgtacggggcgtggcgcggggctcgccgtgccgggcggggggtggcggcaggtgggggtgccgggcggggcggggccgcctcgggccggggagggctcgggggaggggcgcggcggcccccggagcgccggcggctgtcgaggcgcggcgagccgcagccattgccttttatggtaatcgtgcgagagggcgcagggacttcctttgtcccaaatctgtgcggagccgaaatctgggaggcgccgccgcaccccctctagcgggcgcggggcgaagcggtgcggcgccggcaggaaggaaatgggcggggagggccttcgtgcgtcgccgcgccgccgtccccttctccctctccagcctcggggctgtccgcggggggacggctgccttcgggggggacggggcagggcggggttcggcttctggcgtgtgaccggcggctcttgagcctctgctaaccatgttcatgccttcttctttttcctacagcttcgaacctgggcaacgtgctggttattgtgctgtctcatcattttggcaaaatcgattgaattctggccaagtggatccgctagctctagagtcgacggtaccagtactaagcttgcctcgaggatatcccatggagatctatggggacatcatgaagccccttgagcatctgacttctggctaataaaggaaatttattttcattgcaatagtgtgttggaattttttgtgtctctcactcggaaggacatatgggagcatgccctaggcagctgtccggaaccggt

SEQ ID NO: 18 - DNA, 768 bp, Artificial sequence
atcgatgccaccatgagccgcctggataagtccaaagtgatcaactctgccctggagctgctgaatggagtgggaatcgagggactgaccacaaggaagctggcacagaagctgggagtggagcagcctaccctgtactggcacgtgaagaacaagcgcgccctgctggacgcactgccaatcgagatgctggatcggcaccacacacacagctgcccactggagggagagtcctggcaggattttctgcggaacaatgccaagtcttatagatgtgcactgctgagccacagggacggagcaaaggtgcacctgggaaccaggcccacagagaagcagtacgagaccctggagaaccagctggccttcctgtgccagcagggcttttccctggagaatgccctgtatgccctgtctgccgtgggccactttaccctgggatgcgtgctggaggagcaggagcaccaggtggccaaggaggagagagagacaccaaccacagatagcatgccccctctgctgaagcaggccatcgagctgttcgacaggcagggagcagagccagccttcctgtttggcctggagctgatcatctgcggcctggagaagcagctgaagtgtgagtccggaggacctacagacgcactggacgatttcgacctggatatgctgccagccgatgccctggacgattttgacctggatatgctgcccgccgacgccctggatgactttgacctggacatgctgcctggctgataactcgag

SEQ ID NO: 19 - DNA, 765 bp, Artificial sequence
atcgatgccaccatgtccagactggacaagagcaaagtcataaacggcgctctggaattactcaatggagtcggtatcgaaggcctgacgacaaggaaactcgctcaaaagctgggagttgagcagcctaccctgtactggcacgtgaagaacaagcgggccctgctcgatgccctgccaatcgagatgctggacaggcatcatacccacttctgccccctggaaggcgagtcatggcaagactttctgcggaacaacgccaagtcattccgctgtgctctcctctcacatcgcgacggggctaaagtgcatctcggcacccgcccaacagagaaacagtacgaaaccctggaaaatcagctcgcgttcctgtgtcagcaaggcttctccctggagaacgcactgtacgctctgtccgccgtgggccactttacactgggctgcgtattggaggaacaggagcatcaagtagcaaaagaggaaagagagacacctaccaccgattctatgcccccacttctgagacaagcaattgagctgttcgaccggcagggagccgaacctgccttccttttcggcctggaactaatcatatgtggcctggagaaacagctaaagtgcgaaagcggcgggccggccgacgcccttgacgattttgacttagacatgctcccagccgatgcccttgacgactttgaccttgatatgctgcctgctgacgctcttgacgattttgaccttgacatgctccccgggtaactcgag

SEQ ID NO: 20 - DNA, 1320 bp, Artificial sequence
ctcgaggcccctctccctcccccccccctaacgttactggccgaagccgcttggaataaggccggtgtgcgtttgtctatatgttattttccaccatattgccgtcttttggcaatgtgagggcccggaaacctggccctgtcttcttgacgagcattcctaggggtctttcccctctcgccaaaggaatgcaaggtctgttgaatgtcgtgaaggaagcagttcctctggaagcttcttgaagacaaacaacgtctgtagcgaccctttgcaggcagcggaaccccccacctggcgacaggtgcctctgcggccaaaagccacgtgtataagatacacctgcaaaggcggcacaaccccagtgccacgttgtgagttggatagttgtggaaagagtcaaatggctctcctcaagcgtattcaacaaggggctgaaggatgcccagaaggtaccccattgtatgggatctgatctggggcctcggtgcacatgctttacatgtgtttagtcgaggttaaaaaaacgtctaggccccccgaaccacggggacgtggttttcctttgaaaaacacgatgataatatggccacaaccatggtgagcaagggcgaggagctgttcaccggggtggtgcccatcctggtcgagctggacggcgacgtaaacggccacaagttcagcgtgtccggcgagggcgagggcgatgccacctacggcaagctgaccctgaagttcatctgcaccaccggcaagctgcccgtgccctggcccaccctcgtgaccaccctgacctggggcgtgcagtgcttcagccgctaccccgaccacatgaagcagcacgacttcttcaagtccgccatgcccgaaggctacgtccaggagcgcaccatcttcttcaaggacgacggcaactacaagacccgcgccgaggtgaagttcgagggcgacaccctggtgaaccgcatcgagctgaagggcatcgacttcaaggaggacggcaacatcctggggcacaagctggagtacaactacatcagccacaacgtctatatcaccgccgacaagcagaagaacggcatcaaggccaacttcaagatccgccacaacatcgaggacggcagcgtgcagctcgccgaccactaccagcagaacacccccatcggcgacggccccgtgctgctgcccgacaaccactacctgagcacccagtccgccctgagcaaagaccccaacgagaagcgcgatcacatggtcctgctggagttcgtgaccgccgccgggatcactctcggcatggacgagctgtacaagtaaagatct

SEQ ID NO: 21 - DNA, 1044 bp, Artificial sequence
ggatccgccaccatgggcaagtccaaggagatctctcaggacctgagaaagaggatcgtggatctgcacaagagcggcagctccctgggagcaatctccaagcgcctggcagtgcctcggtctagcgtgcagaccatcgtgcgcaagtacaagcaccacggcaccacacagccttcttatcggagcggccggagaagggtgctgagcccacgcgacgagcggacactggtgcgcaaggtgcagatcaacccccggaccacagccaaggatctggtgaagatgctggaggagaccggcacaaaggtgtccatctctaccgtgaagagagtgctgtacaggcacaacctgaagggccactccgccagaaagaagcctctgctgcagaataggcacaagaaggcaaggctgaggttcgcaaccgcacacggcgacaaggatcgcacattttggcggaacgtgctgtggtctgacgagaccaagatcgagctgttcggccacaatgatcacagatacgtgtggaggaagaagggcgaggcctgcaagcccaagaataccatccctacagtgaagcacggaggaggctccatcatgctgtggggatgttttgcagcaggaggaacaggcgccctgcacaagatcgacggcatcatggatgccgtgcagtatgtggacatcctgaagcagcacctgaagacctctgtgagaaagctgaagctgggcaggaagtgggtgttccagcacgacaacgatccaaagcacacaagcaaggtggtggccaagtggctgaaggacaataaggtgaaggtgctggagtggcccagccagtcccctgatctgaacccaatcgagaatctgtgggccgagctgaagaagagagtgagggcccggagacccaccaacctgacacagctgcaccagctgtgccaggaggagtgggccaagatccacccaaattactgtggcaagctggtggagggctatcccaagaggctgacccaggtgaagcagtttaagggcaacgccacaaagtattgataactcgag

SEQ ID NO: 22 - DNA, 376 bp, Artificial sequence
acgcgtgacgaggatcgttcgagcgagtttactccctatcagtgatagagaacgtatgtcgagtttactccctatcagtgatagagaacgatgtcgagtttactccctatcagtgatagagaacgtatgtcgagtttactccctatcagtgatagagaacgtatgtcgagtttactccctatcagtgatagagaacgtatgtcgagtttatccctatcagtgatagagaacgtatgtcgagtttactccctatcagtgatagagaacgtatgtcgaggtaggcgtgtacggtgggaggcctatataagcaaccggtgtttagtgaaccgtcagatctacaaacagaccagattgtctgtttgttttcgaaatcgat

SEQ ID NO: 23 - DNA, 344 bp, Artificial sequence
tccctatcagtgatagagaacgtatgaagagtttactccctatcagtgatagagaacgtatgcagactttactccctatcagtgatagagaacgtataaggagtttactccctatcagtgatagagaacgtatgaccagtttactccctatcagtgatagagaacgtatctacagtttactccctatcagtgatagagaacgtatatccagtttactccctatcagtgatagagaacgtattaggcgtgtacggtgggcgcctataaaagcagagctcgtttagtgaaccgtcagatcgcctggagcaattccacatacaaacagaccagattgtctgtttgtt

SEQ ID NO: 24 - DNA, 19 bp, Artificial sequence
tccctatcagtgatagaga

SEQ ID NO: 25 - DNA, 28 bp, Artificial sequence
taggcgtgtacggtgggcgcctataaaa

SEQ ID NO: 26 - DNA, 29 bp, Artificial sequence
taggcgtgtacggtgggaggcctatataa

SEQ ID NO: 27 - DNA, 28 bp, Artificial sequence
tacaaacagaccagattgtctgtttgtt

SEQ ID NO: 28 - DNA, 324 bp, Artificial sequence
tccctatcagtgatagagaacgtatgaagagtttactccctatcagtgatagagaacgtatgcagactttactccctatcagtgatagagaacgtataaggagtttactccctatcagtgatagagaacgtatgaccagtttactccctatcagtgatagagaacgtatctacagtttactccctatcagtgatagagaacgtatatccagtttactccctatcagtgatagagaacgtattaggcgtgtacggtgggcgcctataaaagcagagctcgtttagtgaaccgtcagatacaaacagaccagattgtctgtttgtt

SEQ ID NO: 29 - DNA, 332 bp, Artificial sequence
tccctatcagtgatagagaacgtatgtcgagtttactccctatcagtgatagagaacgatgtcgagtttactccctatcagtgatagagaacgtatgtcgagtttactccctatcagtgatagagaacgtatgtcgagtttactccctatcagtgatagagaacgtatgtcgagtttatccctatcagtgatagagaacgtatgtcgagtttactccctatcagtgatagagaacgtatgtcgaggtaggcgtgtacggtgggaggcctatataagcaaccggtgtttagtgaaccgtcagatctacaaacagaccagattgtctgtttgtt

SEQ ID NO: 30 - DNA, 352 bp, Artificial sequence
tccctatcagtgatagagaacgtatgtcgagtttactccctatcagtgatagagaacgatgtcgagtttactccctatcagtgatagagaacgtatgtcgagtttactccctatcagtgatagagaacgtatgtcgagtttactccctatcagtgatagagaacgtatgtcgagtttatccctatcagtgatagagaacgtatgtcgagtttactccctatcagtgatagagaacgtatgtcgaggtaggcgtgtacggtgggaggcctatataagcaaccggtgtttagtgaaccgtcagatcgcctggagacgccatcataatacaaacagaccagattgtctgtttgtt

SEQ ID NO: 31 - DNA, 488 bp, Artificial sequence
tcccggccgggaacggtgcattggaacgcggattccccgtgccaagagtgacgtaagtaccgcctatagagtctataggcccacaaaaaatgctttcttcttttaatatacttttttgtttatcttatttctaatactttccctaatctctttctttcagggcaataatgatacaatgtatcatgcctctttgcaccattctaaagaataacagtgataatttctgggttaaggcaatagcaatatttctgcatataaatatttctgcatataaattgtaactgatgtaagaggtttcatattgctaatagcagctacaatccagctaccattctgcttttattttatggttgggataaggctggattattctgagtccaagctaggcccttttgctaatcatgttcatacctcttatcttcctcccacagctcctgggcaacgtgctggtctgtgtgctggcccatcactttggcaaagaattggga

SEQ ID NO: 32 - DNA, 31 bp, Artificial sequence
tcaggatccatctgcgatctaagtaagcttg

SEQ ID NO: 33 - DNA, 29 bp, Artificial sequence
tcaactcgagctagaattacacggcgatc

SEQ ID NO: 34 - DNA, 27 bp, Artificial sequence
gtcaatcgatggagtcgctgcgcgctg

SEQ ID NO: 35 - DNA, 29 bp, Artificial sequence
gtcggatccctgtaggaaaaagaagaagg

SEQ ID NO: 36 - DNA, 26 bp, Artificial sequence
gtcaatcgatgtaagtgccgtgtgtg

SEQ ID NO: 37 - DNA, 30 bp, Artificial sequence
gtcggatccctgaaatggaagaaaaaaact

SEQ ID NO: 38 - DNA, 30 bp, Artificial sequence
gtcaatcgatgtaagtatcaaggttacaag

SEQ ID NO: 39 - DNA, 25 bp, Artificial sequence
gtcggatccctgtggagagaaaggc